European Patent Application EP 4 176 890 A1, published May 10, 2023. Title: OXYTOCIN-MIMETIC COMPOSITIONS AND USES THEREOF. Applicant: INSERM (Institut National de la Santé et de la Recherche Médicale) UNIVERSITÉ DE ROUEN TARGEDYS. The sequence listing filed with the application follows.

SEQUENCE LISTING (44 sequences)

SEQ ID NO: 1 - protein, 395 aa, Lactobacillus salivarius
  elongation factor tu
MAKEHYERTKPHVNIGTIGHVDHGKTTLTAAITKVLAEKGLAEASDYASIDAAPEERERGITINTAHVEYETEKRHYAHIDAPGHADYVKNMITGAAQMDGAILVVAATDGPMPQTREHILLARQVGVEYIVVFLNKCDLVDDDELLDLVEMEVRDLLSEYDFPGDDIPVIRGSALKALEGDKDAEAQIMELMDTVDEYIPTPQRPTDKPFLMPVEDVFTITGRGTVASGRIDRGTVKVGDEVEIVGLKDDVVKTTVTGVEMFRKTLDEGEAGDNIGALLRGVDRTQVERGQVLAKPGSIQTHKKFKGEVYVLTKDEGGRHTPFFSNYRPQFYFHTTDVTGVIELPEGVEMVMPGDNVTFTVELIAPVAIEKGLKFTVREGGRTVGAGVVSEIDD

SEQ ID NO: 2 - protein, 450 aa, Lactobacillus salivarius
  glucose-6-phosphate isomerase
MAHISFDSSNLTKFVNDNELGEMQALVTAVDKELREGTGAGNDFRGFLNLPVDYDKDEFDRIKKAAKKIQSDSEVLVVIGIGGSYLGARAAIDFLHHQFFNLLPAEKRNAPQIFFAGNSISGSYVHDLIELIGDRDFSVNVISKSGTTTEPSIAFRVFKEKLIAKYGVEGARERIYATTDRARGALKTEADAEGYETFVIPDDVGGRFSVLTPVGLLPIAVSGADIDKLMQGAADAREEYSDADLTKNEAYQYAALRNILYRKGYTTEILENYEPTLQYFAEWWKQLMGESEGKDGKGIYPSSANFSTDLHSLGQYIQEGMRNLMETVITVGNPTNDTDIPKEEENLDGLGYLEGKSMNYVNSKAFQGVVLAHTDGNVPNMIVNIPDQTEYTLGYMIYFFEIAVAISGYLNGINPFNQPGVEAYKKNMFALLGRPGYEELTKELQDRLNK

SEQ ID NO: 3 - protein, 400 aa, Lactobacillus salivarius
  Phosphoglycerate kinase
MAKLIVSDLDVKGKKVLMRVDFNVPIKNGVIGNDNRIVAALPTINYIIEHDGKAILFSHLGRIKKEEDKKELSLRPVAERLAELLNKPVTFVPATRGAQLEDAINNMNDGDVLLVENTRFEDLDGKKESGNDPELGKYWASLGDVFVNDAFGTAHRSHASNVGISEAMKAEGKQAAAGYLLEKEIKFLGNAVDSPKHPFVAILGGAKVSDKIGVINHLLGKADKVIVGGGMTYTFYAAKGIKIGNSLVEKDKIELAKEIMEKAGDKLVLPVDNVCAKEFNNDAPSEVVEGDIPDGYMALDIGPKSVELFEDTLKDAKTVVWNGPMGVFEMSNFAKGTLEVGKFLGTLSDATTIVGGGDSTAAVQQLGVADKLTHISTGGGASLEYLEGKTLPGIAAVSDK

SEQ ID NO: 4 - protein, 396 aa, Lactobacillus gasseri
  elongation factor tu
MAEKEHYERTKPHVNIGTIGHVDHGKTTLTAAITTVLAEDGLAQAEDYSQIDAAPEEKERGITINTAHVEYETKNRHYAHMDAPGHADYIKNMITGAAQMDGAILVVAATDGPMPQTREHILLARQVGVKYIVVFLNKVDLVDDPELIDLVEMEVRDLLTEYDYPGDDVPVIRGSALKALQGDPEQQDVIRKLMETVDEYIPTPERDTDKPFLMPVEDVFTITGRGTVASGRIDRGTVKVGDEVEIVGLTDKVEKSTVTGLEMFHKTLDLGEAGDNVGVLLRGIDRDQVERGQVLAAPGSIQTHKKFKGQVYILNKDEGGRHTPFFSDYRPQFYFHTTDVTGKIELPEGTEMVMPGDNVEFTVELIKPVAIEKGTKFTIREGGKTVGAGQVTEILD

SEQ ID NO: 5 - protein, 447 aa, Lactobacillus gasseri
  Glucose-6-phosphate isomerase
MSKVVHFDASKLTPFVHENELKEMQAMVTAADQELREGTGAGSDFRGWIDLPINYDKDEFDRIKKAAKKIQNDSEVLVGIGIGGSYLGAQASIEFLNSSFYGREKEKYPTVVFCGNSLSGSYLYDLLEWLGDKDFSINIISKSGTTTEPSIAFRVLKDKLIKKYGKEEAAKRIYATTDRAKGALKTEADAEGYEEFVVPDDIGGRFSVLSAVGLLPIAVAGGDIDAMMKGAADARAAYTDPDVSKDNPYQYAALRNILYRKGYTTELLENYEPSLRMFGEWWKQLMGESEGKDQKGIYPSSANFTTDLHSLGQYIQEGRRNLMETVIRVESPEHDVTIPDDKENLDQLNFLSGKTMNYVNDRAYEGVVLAHTDGGVPVMTVDIENQSAHTLGYLIYWFELAVGISGYLNGINPFNQPGVESYKRNMFGLLNKPGYEDLHDDLTKRLK

SEQ ID NO: 6 - protein, 403 aa, Lactobacillus gasseri
  Phosphoglycerate kinase
MAKLIVSDLDLKGKKVLVRVDFNVPIKNGVIGDDNRIVAALPTIKYIIEHGGKAILLSHLGRVKSDADKKELSLRPVAERLSELLKKPVTFVPENEGKEVEETIDKMKDGDVIVLENTRFQDIDNDFGKRESKNDPKLGEYWASLGDVFVNDAFGTAHRSHASNVGIATAMKKAGKPAAAGFLLEKEIKFLGDAVENPVHPFVTILGGAKVSDKIGVIENLIPKSDHILIGGGMAYTFLAAQGHKIGKSLFEADKVELAKELLAKAGDKIVLPVDNVAATEFSNDAPHEVVGDDIPDNEMGLDIGPKTVEKFRDILKDAKTVVWNGPMGAFEMPNYAEGTLEVGRALADLKDAVTIIGGGDSTAAAKQLGIAPKISHISTGGGASLNYLEGKELPGIACVSDK

SEQ ID NO: 7 - protein, 428 aa, Lactobacillus gasseri
  enolase1
MLKSVIENVHALEIFDSRGNPTVEVFVTLSNGVVGKAEVPSGASTGENEAVELRDGGSRLGGKGVMNAVNNVNTEINDALKGLDPHDQPNIDATMIALDGTPNKGRLGANAILGVSMATACAAAKDNHQPLYRYLGGTDLEMPQTFHNVINGGEHADNGIDIQEFMITPVAKTSFRDGFEKIVNVYHTLKKVLEDMGYETGLGDEGGFAPNMKNSEEALKALHESIIKAGYKPGEDIAIACDCAASYFYNKEDGKYHLEGKVLTDEELADYYDKLLDEFPELISMEDPYDENDVEGMVKFTESHKDRIQIVLDDFICTNPKLLNKAIHEGAGNASLIKLNQIGTVTETLETIRLSRKNGYNTMISHRSGETGDTFIADFAVAVNGGQLKSGAPARSERVEKYNRLLEIEEELGKGERLAFFPDNVDLD

SEQ ID NO: 8 - protein, 432 aa, Lactobacillus gasseri
  enolase2
MSVITDIHAREVLDSRGNPTVEAEVYTELGGFGRAIVPSGASTGEHEAVELRDGDKSRFGGQGVLTAVENVNGEIAKAVIGLDVTDQRLIDQTMIDLDGTPNKGRLGANAILSVSLASARAAADELGLPLYEYLGGPNAHVLPTPMMNVINGGKHADNNVDIQEFMIMPVGAKSLHEAVRMGAETFHTLKGLLQERGESTAVGDEGGFAPNLKNNEEPFEILVEAIQRAGYKPGQDIAIAFDCAASEFYNKDTKKYVTVADGREYTAEEWTSLIEDLVDKYPVISVEDPLDENDWEGWKTFTERLGDKVQIVGDDLFVTNTSYLEKGIKMGVANSILIKLNQIGTLTETFEAIEMAKEAGYTAVVSHRSGETEDTTIADLVVATNAGQIKTGSMSRTDRIAKYNQLMRIEEALGSTAQYKGIHSFYNLHKQF

SEQ ID NO: 9 - protein, 396 aa, Lactobacillus camelliae
  elongation factor tu
MAEKEHYERTKPHVNIGTIGHVDHGKTTLTAAITKVLAAKGLAKEQDYASIDAAPEEKERGITINTAHVEYETEKRHYAHIDAPGHADYVKNMITGAAQMDGAILVVAATDGPMPQTREHILLARQVGVDYIVVFLNKTDLVDDDELIDLVEMEVRELLSEYDFPGDDIPVIRGSALKALQGDPEQEKVIQELMDTVDEYIPTPVRDTDKPFLMPVEDVFTITGRGTVASGRIDRGTVKIGDEVEIVGLHDEVLKSVVTGLEMFRKTLDLGEAGDNVGILLRGINRDQVERGQVLAKPGSIQTHKKFKAEVYILTKEEGGRHTPFFSNYRPQFYFHTTDVTGVIELPDGVEMVMPGDNVTFEVDMIAPVALEKGTKFTVREGGRTVGAGVVSEILG

SEQ ID NO: 10 - protein, 286 aa, Lactobacillus camelliae
  Fructose tagatose bisphosphate aldolase
MFQAARKGHYAIGAFNTNNLEWTRALLKGAQELNVPILIQTSMGAAKYMGGYKLCKALIELEAESMNITVPVVIHLDHGNFEAAKEAIAAGYNSVMFDGHDLPFDENLEKTKEIVKLAHAKGISVEAEVGSIGGEEDGVIGEGELASVEEAKTLAATGIDFMAAGIGNIHGKYPSNWKGLHFDRLQEIADAVDLPLVLHGGSGIPQDQVEKAISMGIAKLNINTECQLAFAKATREYILANKDQEGKGYDPRKLLAPGTQAITDTFKEISGWMGTRPVKMVPEEIK

SEQ ID NO: 11 - protein, 290 aa, Lactobacillus camelliae
  2,5-didehydrogluconate reductase
MAEISKMSDTYTLSNGVKIPIVGFGTWQTPDGDVAKHSVEVAIKDGYRHIDTAAMYRNEDSVGEGIKAGLAAAGLKRDDLFVTTKLNNNAHSFDLVQKAIDESLTKLGLDHVDLYLIHWPNPVSFRDSYPDSLKETWRGMEQVYKDGKARAIGISNFRQAHLDVIKADATVEPMVNQIFLNPSDLQPAVTKMNAENNILSEAYSPLGTGKLLGNEELAKVAAKYGKGVAQVLLRWSLQHGFLPLAKSVHDARIKENTELFDFTLSDEDMKTLDGMRGVAGLATDPDTTNF

SEQ ID NO: 12 - protein, 246 aa, Lactobacillus camelliae
  Triosephosphate isomerase
MAGNWKMNKNPEETQAFLDGVKGKLPESSKVQTVIAAPAIDLTTLVAGAKGTPLQTAAENCYFEDAGAFTGETSPKALKDMGLDYVVIGHSERRGYFHETDQDINKKAKAILKNGLLPIICCGESLDQREAGQTNDWVASQVEAALAGISAADVKNSVIAYEPIWAIGTGKTASADQAQEVVAHIRSIVAKLYDAETADAVRILYGGSVKPANVKELMAKPDIDGGLVGGASMDPESFVALANYQD

SEQ ID NO: 13 - protein, 230 aa, Lactobacillus camelliae
  2,3-bisphosphoglycerate-dependent phosphoglycerate mutase
MAKLVLIRHGQSEWNLSNQFTGWVDVDLSEKGTEEAKEAGRRIKKAGLEFDQAYTSVLTRAIKTLHYALEESDQLWIPETKTWRLNERHYGALQGQNKAEAAKKWGDEQVHIWRRSYDTLPPLLSADDEGSAAKDRRYANLDPRIIPGGENLKVTLERVIPFWEDHIAPDLLDGKNVIIAAHGNSLRALTKYIENISDEDIINLEMTTGEPVVYTFNDKLEVTDKVKLSK

SEQ ID NO: 14 - protein, 395 aa, Lactobacillus plantarum [sequence omitted]

SEQ ID NO: 15 - protein, 518 aa, Lactobacillus plantarum
  GMP synthase
MAKTDTASFDSILVLDFGSQYNQLITRRIRDFGVYSELLPNTITAEEIKARHPKGIIFSGGPNSVYDDGAFRVDPEIFKLGLPILGICYGMQLMTYTLAGGKVESADNREYGKANIDVTSDSATLFKDTPAEQSVWMSHGDLVTQAPDGFDVVATSKNCPIAAIQDVDRKLYGIQFHAEVRNTDYGNDILRHFAFDVCQAEANWSMDDFIDMQIEKIRAEVGDKKVLLGLSGGVDSSVVGVLLHKAIGTQLTSIFVDHGLLRKGEADQVMASLEGKFGLNIIKVDAKDRFLSKLAGVSDPERKRKIIGNEFIQVFDEEATKLNGMEFLAQGTLYTDVIESGTSTAQTIKSHHNVGGLPEDMQFKLIEPLRTLFKDEARELGEKLGMPSDLVWRQPFPGPGLGIRVIGEITEDKLEIVRDSDFILRDEIKKAGLDREIWQYFTVLPGIKSVGVMGDGRTYDYTVGIRAVTSIDGMTADFARIPWDVLQKISVRIVNEVDHVNRIVYDVTSKPPSTIEWE

SEQ ID NO: 16 - protein, 605 aa, Lactobacillus plantarum
  Glutamine-fructose-6-phosphate aminotransferase
MCGIVGVTGKDSAVSILLNGLEKLEYRGYDSAGIYVNDQDGHDYLVKEKGRIDDLRKEVGEAVHGSTGIGHTRWATHGEPSVANAHPQVSADGRFYLVHNGVIENFEDLKQTYLSDVTFKSQTDTEVIVQLVDRFVTKEGLSTLAAFRKTLGLLGHSSYGFLLMDKEDPDTLYVAKNKSPLLIGVGEGFNVVCSDSLAMLDQTKDFLELHDGEIVVVKPDEIKITNQAGEPVERKPFHVDIDAAQADKGTYPFYMLKEIDEQPNVMRKLSQVYLNDAGDPIINDDLLTALKAADRLYIVAAGTSYHAGLVGAKLFESLANVPTEVHVSSEFAYNQPLLSAHPFFIFLTQSGETADSREVLLNVNDQHFPSLTITNVPNSTLSREATYTLLLHAGPEIAVASTKAYTAQIALQAILAKALGVAVDQPAATAFDVKQQLALVANGMQSLVDEKATFEKIAKSALLNTPNAFYIGRGLDYAVSLETALKLKEISYVQAEGFASGELKHGTIALIEKDTPVIGIITQKNTAGLTRSNLQEVAARGAKTVTIVTDSLAKDGDTVILPTVDERLTALLSVVPGQLLAYYTSLNKGLDVDKPRNLAKSVTVE

SEQ ID NO: 17 - protein, 396 aa, Lactobacillus reuteri
  Elongation factor Tu
MAEKEHYERTKPHVNIGTIGHVDHGKTTLTAAITKVLAAKGLAKAEDYADIDAAPEEKERGITINTAHVEYETEKRHYAHIDAPGHADYVKNMITGAAQMDGAILVVAATDGPMPQTREHILLARQVGVQYIVVFLNKTDLVDDDELVDLVEMEVRDLLSEYDFPGDDVPVVRGSALKALEGDPEQEKVILHLMDVIDDYIPTPKRPTDKPFMMPVEDVFTITGRGTVASGRIDRGTVKVGDEVEIVGLTEDVLKSTVTGLEMFHKTLDLGEAGDNVGVLLRGISHDQIQRGQVLAEPGSIQTHKNFKGEVYVMTKEEGGRHTPFFSNYRPQFYFHTTDVTGTIELPDGVEMVMPGDNVTFTVNLQKPVALEKGLKFTIREGGHTVGAGVVSDILD

SEQ ID NO: 18 - protein, 452 aa, Lactobacillus reuteri
  Glucose-6-phosphate isomerase
MTHIKFDSSALKQFVHENELGEMQAMVNAANDELRNGTGAGADFRDWLHLPTEYDKEEFARIKKAADKIQRDSDVLVVIGIGGSYLGAQMAIDFLHNTFYQAQNAKDRKAPLVVFAGNSLSSTYVHDLIQLIGDKDFSINVVSKSGTTTEPSIAFRIFKGLLIKKYGENEANKRIYATTDKTKGALKTEADAHGYETFVIPDGVGGRYSVLSAVGLLPIAASGADIDKLMEGAAQAEKDYVDPDLTKNEAYQYAAYRNILYRKGYETELLENYEPNMRMFAEWWKQLAGESEGKDQKGIYPSSANFTTDLHSLGQYIQEGRRFLMETVVKLDKPNYDMEIPTEPDNLDGLGYLEGKTMDYVNTKAYEAVVAAHTDGGVPVMTVHIPQEDEYTLGYLIYFFEVAMGISGYLNGINPFNQPGVEAYKTNMFGLLGKPGYEEIGKELRAKMDKND

SEQ ID NO: 19 - protein, 401 aa, Bifidobacterium dentium
  Phosphoglycerate kinase
MKTLKDLGDLKGKRVLVRADFNVPLDGTTITDDGRIKAALPTIKALREEGAKVILMAHLGRPKGKVVPELSLAPVATRLGELLGVEVPLASDTYGEDAQAKVAAMNDGDVVLLQNVRFNPEETSKDPEERAAYAKKIAALGEAFVSDGFGVVHRAQGSNYDVAADLPAAAGLLVEKEVKALSRATVDPERPLTVVLGGSKVSDKLGVIENLLDKADRLVIGGGMVYTFLKAKGLEVGTSLLEEDQVETVKGYIERAEKNGVELVLPTDIVVNPVFPKSDEDIAPEVVAADAIPADKMGLDIGPDSQKLFHDKIVDSKTVVWNGPMGVFEVPAFAAGTEAVAQGLVDATAAGAFTIVGGGDSASAVRNLGFPEDGFSHISTGGGASLEFLEGKELPGLKVLD

SEQ ID NO: 20 - protein, 825 aa, Bifidobacterium dentium
  phosphoketolase
MTSPVIGTPWKKLNAPVSEEAIEGVDKYWRAANYLSIGQIYLRSNPLMKEPFTREDVKHRLVGHWGTTPGLNFLIGHINRLIADHQQNTVIIMGPGHGGPAGTAQSYLDGTYTEYFPNITKDEAGLQKFFRQFSYPGGIPSHYAPETPGSIHEGGELGYALSHAYGAVMNNPSLFVPAIVGDGEAETGPLATGWQSNKLVNPRTDGIVLPILHLNGYKIANPTILSRISDEELHEFFHGMGYEPYEFVAGFDNEDHLSIHRRFAELFETVFDEICDIKAAAQTDDMTRPFYPMIIFRTPKGWTCPKFIDGKKTEGSWRSHQVPLASARDTEAHFEVLKNWLESYKPEELFDANGAVKPEVTAFMPTGELRIGENPNANGGRIREELNLPALEDYEVKEVAEYGHGWGQLEATRRLGVYTRDIIKNNPDSFRIFGPDETASNRLQAAYDVTNKQWDAGYLSAQVDEHMAVTGQVTEQLSEHQMEGFLEAYLLTGRHGIWSSYESFVHVIDSMLNQHAKWLEATVREIPWRKPISSMNLLVSSHVWRQDHNGFSHQDPGVTSVLLNKCFNNDHVIGIYFPVDSNMLLAVAEKCYKSTDMINAIIAGKQPAATWLTLDEARAELEKGAAEWEWASTAKSNDEAQIVLASAGDVPAQEIMAAADKLDAMGIKFKVVNVVDLVKLQSTKENDEAISDADFADLFTEDKPVLFAYHSYARDVRGLIYDRPNHDNFNVHGYEEQGSTTTPYDMVRVNNIDRYELVAEALRMIDADKYADKIDELEAFRKEAFQFAVDNGYDHPDYTDWVYSGVNTNKQGAVSATAATAGDNE

SEQ ID NO: 21 - protein, 399 aa, Bifidobacterium pseudolongum subsp. pseudolongum
  Elongation factor Tu
MAKEKYERTKPHVNIGTIGHVDHGKTTLTAAISKVLHDEFPDLNPEYDFNQIDAAPEEQQRGITINIAHIEYQTEKRHYAHVDCPGHADFVKNMITGAAQMDGAILVVAATDGPMAQTREHVLLARQVGVPKILVALNKCDMVDDEELIELVEEEVRDLLDENGFDRDCPVVHTSAYGALHDDAPDHEKWVETVKELMNDVDDYIPTPVHDLDKPFLMPIEDVFTISGRGTVVTGRVERGKLPINTNVEIVGIRPTQTTTVTSIETFHKQMDECEAGDNTGLLLRGLGRTDVERGQVVAAPGSVTPHTKFEGEVYVLTKDEGGRHSPFFSNYRPQFYFRTTDVTGVITLPEGVEMVQPGDHATFTVELIQPIAMEEGLTFAVREGGHTVGSGRVTKILA

SEQ ID NO: 22 - protein, 401 aa, Bifidobacterium pseudolongum subsp. pseudolongum
  phospoglycerate kinase
MKTLKDLGDLKGKRVLVRADFNVPLDGTTITDDGRIKAALPTIEELRKDGAKVILMAHLGRPKGKVVPELSLAPVAKRLSELLGCDVVLASDTYGPDAQTKVAAMNDGDVVLLENVRFNPEETSKDEAERAAYAKKIAALGDVFVSDGFGVVHRAQGSNYDVAADLPAAAGLLVEKEVKALSKATENPERPFTVVLGGSKVSDKLGVIENLLDKADRLVIGGGMVFTFLKAKGYEVGTSLLEEDQIDKVKGYIETAEKNGVELVLPVDIVVNKGFPAGDTPIDPQVVPADQIPSDMMGLDIGPESCKLFHDKIVDSKTVVWNGPMGVFEIPQFANGTRAVAQALVDATANGAFTIVGGGDSAAAVRNLGFPEDGFSHISTGGGASLEFLEGKELPGLKVLD

SEQ ID NO: 23 - protein, 401 aa, Bifidobacterium pseudolongum subsp. globosum
  Phosphoglycerate kinase
MKTLKDLGDLKGKRVLVRADFNVPLDGTTITDDGRIKAALPTIEELRKDGAKVILMAHLGRPKGKVVPELSLAPVAKRLSELLGCDVVLASDTYGPDAQAKVAAMNDGDVVLLENVRFNPEETSKDEAERAEYAKKIAALGDVFVSDGFGVVHRAQGSNYDVAADLPAAAGLLVEKEVKALSKATENPERPFTVVLGGSKVSDKLGVIENLLDKADRLVIGGGMVFTFLKAKGYEVGTSLLEEDQIDKVKGYIETAEKNGVELVLPVDIVVNKGFPAGDTPIDPQVVPADQIPSDMMGLDIGPESCKLFHDKIVDSKTVVWNGPMGVFEIPQFANGTRAVAQALVDATANGAFTIVGGGDSAAAVRNLGFPEDGFSHISTGGGASLEFLEGKELPGLKVLD

SEQ ID NO: 24 - protein, 825 aa, Bifidobacterium pseudolongum subsp. globosum
  Probable phosphoketolase
MTNPVIGTPWQKLDRPVSEEAIEGMDKYWRVTNYMSIGQIYLRSNPLMKEPFTRDDVKHRLVGHWGTTPGLNFLLAHINRLIADHQQNTVFIMGPGHGGPAGTSQSYVDGTYTEYYPNITKDEAGLQKFFRQFSYPGGIPSHFAPETPGSIHEGGELGYALSHAYGAVMNNPSLFVPCIIGDGEAETGPLATGWQSNKLVNPRTDGIVLPILHLNGYKIANPTILARISDEELHDFFRGMGYHPYEFVAGFDNEDHMSIHRRFAELFETIFDEICDIKAAAQTDDMTRPFYPMLIFRTPKGWTCPKFIDGKKTEGSWRAHQVPLASARDTEEHFEVLKGWLESYKPEELFNADGSIKDDVTAFMPKGDLRIGANPNANGGVIREDLKLPELDQYEVTGVKEYGHGWGQVEAPRSLGAYCRDIIKNNPDSFRIFGPDETASNRLNATYEVTDKQWDNGYLSSLVDEHMAVTGQVTEQLSEHQCEGFLEAYLLTGRHGIWSSYESFVHVIDSMLNQHAKWLEATVREIPWRKPISSVNLLVSSHVWRQDHNGFSHQDPGVTSVLINKTFNNDHVTNIYFATDANMLLAISEKCFKSTNKINAIFAGKQPAPTWITLDEARAELEAGAAEWKWASNAENNDEVQVVLAAAGDVPTQEIMAASDALNKMGIKFKVVNVVDLLKLQSRENNDEALTDEEFTDLFTADKPVLFAYHSYAQDVRGLIYDRPNHDNFNVVGYKEQGSTTTPFDMVRVNDMDRYALQAAALKMIDADKYADKIDELNAFRQKAFQFAVDNGYDIPEFTDWVYPDVKVDETQMLSATAATAGDNE

SEQ ID NO: 25 - protein, 825 aa, Bifidobacterium ruminantium
  Xylulose-5-phosphate/fructose-6-phosphate phosphoketolase
MTSPVIGTPWKKLNAPVSEEAIEGVDKYWRAANYLSIGQIYLRSNPLMKEPFTREDVKHRLVGHWGTTPGLNFLIGHINRLIADHQQNTVIIMGPGHGGPAGTAQSYLDGTYTEYFPNITKDEAGLQKFFRQFSYPGGIPSHYAPETPGSIHEGGELGYALSHAYGAVMNNPSLFVPAIVGDGEAETGPLATGWQSNKLINPRTDGIVLPILHLNGYKIANPTILSRISDEELHEFFHGMGYEPYEFVAGFDNEDHLSIHRRFAELFETVFDEICDIKAAAQTDDMTRPFYPMIIFRTPKGWTCPKFIDGKKTEGSWRSHQVPLASARDTEAHFEVLKNWLESYKPEELFDENGAVKPEVTAFMPTGELRIGENPNANGGRIREELKLPKLEDYEVKEVAEYGHGWGQLEATRRLGVYTRDIIKNNPDSFRIFGPDETASNRLQAAYDVTNKQWDAGYLSAQVDEHMAVTGQVTEQLSEHQMEGFLEGYLLTGRHGIWSSYESFVHVIDSMLNQHAKWLEATVREIPWRKPISSMNLLVSSHVWRQDHNGFSHQDPGVTSVLLNKCFNNDHVIGIYFPVDSNMLLAVAEKCYKSTNKINAIIAGKQPAATWLTLDEARAELEKGAAEWKWASNVKSNDEAQIVLAATGDVPTQEIMAAADKLDAMGIKFKVVNVVDLVKLQSAKENNEALSDEEFAELFTEDKPVLFAYHSYARDVRGLIYDRPNHDNFNVHGYEEQGSTTTPYDMVRVNNIDRYELQAEALRMIDADKYADKINELEAFRQEAFQFAVDKGYDHPDYTDWVYSGVNTNKQGAVSATAATAGDNE

SEQ ID NO: 26 - protein, 399 aa, Bifidobacterium adolescentis
  Elongation factor Tu
MAKEKYERTKPHVNIGTIGHVDHGKTTLTAAISKVLHEEYPDVNPEYDFNQIDSAPEEAARGITINIAHIEYQTEKRHYAHVDCPGHADFVKNMITGAAQMDGAILVVAATDGPMAQTREHVLLARQVGVPKILVALNKCDMVDDEELIELVEEEVRDLLDENGFDRDCPVIHVSAYGALHDDAPDHEKWVEQVKKLMDAVDDYIPTPVHDLDKPFLMPIEDVFTISGRGTVVTGRVERGKLPVNSNVEIVGIRPTQTTTVTSIETFHKQMDECEAGDNTGLLLRGINRDQVERGQVLAAPGSVTPHTKFEGEVYVLTKDEGGRHSPFFSNYRPQFYFRTTDVTGVITLPEGVEMVQPGDHATFGVELIQPIAMEEGLTFAVREGGHTVGSGRVTKIIE

SEQ ID NO: 27 - protein, 9 aa, Oryctolagus cuniculus
  oxytocin
CYIQNCPLG

SEQ ID NO: 28 - protein, 9 aa, Artificial Sequence
  87-95 position fragment of SEQ ID NO:1
DYVKNMITG

SEQ ID NO: 29 - protein, 9 aa, Artificial Sequence
  13-21 position fragment of SEQ ID NO:2
KFVNDNELG

SEQ ID NO: 30 - protein, 10 aa, Artificial Sequence
  317-326 position fragment of SEQ ID NO:3
KTVVWNGPMG

SEQ ID NO: 31 - protein, 9 aa, Artificial Sequence
  154-162 position fragment of SEQ ID NO:15
ATSKNCPIA

SEQ ID NO: 32 - protein, 9 aa, Artificial Sequence
  371-379 position fragment of SEQ ID NO:16
LTITNVPNS

SEQ ID NO: 33 - protein, 7 aa, Artificial Sequence
  313-319 position fragment of SEQ ID NO:5
QYIQEGR

SEQ ID NO: 34 - protein, 10 aa, Artificial Sequence
  12-21 position fragment of SEQ ID NO:18
KQFVHENELG

SEQ ID NO: 35 - protein, 9 aa, Artificial Sequence
  88-96 position fragment of SEQ ID NO:4
DYIKNMITG

SEQ ID NO: 36 - protein, 12 aa, Artificial Sequence
  160-171 position fragment of SEQ ID NO:8
VDIQEFMIMPVG

SEQ ID NO: 37 - protein, 9 aa, Artificial Sequence
  246-254 position fragment of SEQ ID NO:7
SYFYNKEDG

SEQ ID NO: 38 - protein, 8 aa, Artificial Sequence
  1-8 position fragment of SEQ ID NO:10
MFQAARKG

SEQ ID NO: 39 - protein, 9 aa, Artificial Sequence
  202-210 position fragment of SEQ ID NO:11
AYSPLGTGK

SEQ ID NO: 40 - protein, 8 aa, Artificial Sequence
  61-68 position fragment of SEQ ID NO:12
CYFEDAGA

SEQ ID NO: 41 - protein, 9 aa, Artificial Sequence
  191-199 position fragment of SEQ ID NO:13
KYIENISDE

SEQ ID NO: 42 - protein, 10 aa, Artificial Sequence
  40-49 position fragment of SEQ ID NO:20
IYLRSNPLMK

SEQ ID NO: 43 - protein, 9 aa, Artificial Sequence
  164-172 position fragment of SEQ ID NO:21
GFDRDCPVV

SEQ ID NO: 44 - protein, 9 aa, Artificial Sequence
  89-97 position fragment of SEQ ID NO:21
DFVKNMITG